European Patent Application EP 4 450 512 A1, published October 23, 2024. Title: Production method of oligonucleotides. Applicant: リードファーマ株式会社. The sequence listing filed with the application follows.

SEQUENCE LISTING (9 sequences)

SEQ ID NO: 1 - DNA, 10 bp, synthetic construct
  source 1..10: mol_type = other DNA
tttttttttt

SEQ ID NO: 2 - DNA, 10 bp, synthetic construct
  misc_feature 1..9: note = DNA
  misc_feature 10: note = RNA
  source 1..10: mol_type = other DNA
  modified_base 10: mod_base = OTHER; note = uracil; note = 2'-O-methyl-ribose
tttttttttt

SEQ ID NO: 3 - DNA, 10 bp, synthetic construct
  misc_feature 1..9: note = DNA
  misc_feature 10: note = RNA
  source 1..10: mol_type = other DNA
  modified_base 10: mod_base = OTHER; note = 2'-O, 4'-C-methano-bridged-ribose; note = thymine
tttttttttt

SEQ ID NO: 4 - DNA, 12 bp, synthetic construct
  source 1..12: mol_type = other DNA
ggatgttctcgt

SEQ ID NO: 5 - DNA, 10 bp, synthetic construct
  misc_feature 1..9: note = DNA
  misc_feature 10: note = RNA
  source 1..10: mol_type = other DNA
  modified_base 10: mod_base = OTHER; note = thymine; note = 2'-O-methoxyethyl-ribose
tttttttttt

SEQ ID NO: 6 - DNA, 10 bp, synthetic construct
  misc_feature 1..9: note = DNA
  misc_feature 10: note = RNA
  source 1..10: mol_type = other DNA
  modified_base 10: mod_base = OTHER; note = 2'-O-(2-cyanoethyl)-ribose; note = uracil
tttttttttt

SEQ ID NO: 7 - DNA, 10 bp, synthetic construct
  misc_feature 1..9: note = DNA
  misc_feature 10: note = RNA
  source 1..10: mol_type = other DNA
  modified_base 10: mod_base = OTHER; note = uracil; note = 2'-O-allyl-ribose
tttttttttt

SEQ ID NO: 8 - DNA, 10 bp, synthetic construct
  misc_feature 1..9: note = DNA
  misc_feature 10: note = RNA
  source 1..10: mol_type = other DNA
  modified_base 10: mod_base = OTHER; note = uracil; note = 2'-O-propargyl-ribose
tttttttttt

SEQ ID NO: 9 - DNA, 10 bp, synthetic construct
  misc_feature 1..9: note = DNA
  misc_feature 10: note = RNA
  source 1..10: mol_type = other DNA
  modified_base 10: mod_base = OTHER; note = uracil; note = 2'-O-(3-acetamidopropyl)-ribose
tttttttttt